European Patent Application EP 4 803 885 A1, published September 9, 2026. Title: 一种探针及其在显像和治疗方面的应用. Applicant: 厦门大学. The sequence listing filed with the application follows.

SEQUENCE LISTING (20 sequences)

SEQ ID NO: 1 - protein, 199 aa, synthetic construct
VEEPQNLIKQNCELFEQLGEYKFQNALLVRYTKKVPQVSTPTLVEVSRNLGKVGSKCCKHPEAKRMPCAEDYLSVVLNQLCVLHEKTPVSDRVTKCCTESLVNRRPCFSALEVDETYVPKEFNAETFTFHADICTLSEKERQIKKQTALVELVKHKPKATKEQLKAVMDDFFVEKCCKADDKETCFAEEGKKLVSQLGL

SEQ ID NO: 2 - protein, 199 aa, synthetic construct
KCCADPHECYAKVFDEFKPLVEEPQNLIKQNCELFEQLGEYKFQNALLVRYTKKVPQVSTPTLVEVSRNLGKVGSKCCKHPEAKRMPCAEDYLSVVLNQLCVLHEKTPVSDRVTKCCTESLVNRRPCFSALEVDETYVPKEFNAETFTFHADICTLSEKERQIKKQTALVELVKHKPKATKEQLKAVMDDFFVEKCCKA

SEQ ID NO: 3 - protein, 114 aa, synthetic construct
KTPVSDRVTKCCTESLVNRRPCFSALEVDETYVPKEFNAETFTFHADICTLSEKERQIKKQTALVELVKHKPKATKEQLKAVMDDFFVEKCCKADDKETCFAEEGKKLVSQLGL

SEQ ID NO: 4 - protein, 9 aa, synthetic construct
YPYDVPDYA

SEQ ID NO: 5 - protein, 6 aa, synthetic construct
HHHHHH

SEQ ID NO: 6 - protein, 218 aa, synthetic construct
MSPILGYWKIKGLVQPTRLLLEYLEEKYEEHLYERDEGDKWRNKKFELGLEFPNLPYYIDGDVKLTQSMAIIRYIADKHNMLGGCPKERAEISMLEGAVLDIRYGVSRIAYSKDFETLKVDFLSKLPEMLKMFEDRLCHKTYLNGDHVTHPDFMLYDALDVVLYMDPMCLDAFPKLVCFKKRIEAIPQIDKYLKSSKYIAWPLQGWQATFGGGDHPPK

SEQ ID NO: 7 - protein, 10 aa, synthetic construct
EQKLISEEDL

SEQ ID NO: 8 - protein, 5 aa, synthetic construct
GGGGS

SEQ ID NO: 9 - protein, 10 aa, synthetic construct
GGGGSGGGGS

SEQ ID NO: 10 - protein, 9 aa, synthetic construct
CQDGRMGFC

SEQ ID NO: 11 - protein, 987 aa, synthetic construct [sequence omitted]

SEQ ID NO: 12 - protein, 186 aa, synthetic construct
EETLLNTKLETADLKWVTFPQVDGQWEELSGLDEEQHSVRTYEVCDVQRAPGQAHWLRTGWVPRRGAVHVYATLRFTMLECLSLPRAGRSCKETFTVFYYESDADTATALTPAWMENPYIKVDTVAAEHLTRKRPGAEATGKVNVKTLRLGPLSKAGFYLAFQDQGACMALLSLHLFYKKCAQLTV

SEQ ID NO: 13 - protein, 211 aa, synthetic construct
VEEPQNLIKQNCELFEQLGEYKFQNALLVRYTKKVPQVSTPTLVEVSRNLGKVGSKCCKHPEAKRMPCAEDYLSVVLNQLCVLHEKTPVSDRVTKCCTESLVNRRPCFSALEVDETYVPKEFNAETFTFHADICTLSEKERQIKKQTALVELVKHKPKATKEQLKAVMDDFFVEKCCKADDKETCFAEEGKKLVSQLGLGGGGSQDGRMGF

SEQ ID NO: 14 - protein, 395 aa, synthetic construct
VEEPQNLIKQNCELFEQLGEYKFQNALLVRYTKKVPQVSTPTLVEVSRNLGKVGSKCCKHPEAKRMPCAEDYLSVVLNQLCVLHEKTPVSDRVTKCCTESLVNRRPCFSALEVDETYVPKEFNAETFTFHADICTLSEKERQIKKQTALVELVKHKPKATKEQLKAVMDDFFVEKCCKADDKETCFAEEGKKLVSQLGLGGGGSGGGGSEETLLNTKLETADLKWVTFPQVDGQWEELSGLDEEQHSVRTYEVCDVQRAPGQAHWLRTGWVPRRGAVHVYATLRFTMLECLSLPRAGRSCKETFTVFYYESDADTATALTPAWMENPYIKVDTVAAEHLTRKRPGAEATGKVNVKTLRLGPLSKAGFYLAFQDQGACMALLSLHLFYKKCAQLTV

SEQ ID NO: 15 - protein, 7 aa, synthetic construct
  source 1..7: note = Cyclic peptide
QDGRMGF

SEQ ID NO: 16 - protein, 213 aa, synthetic construct
VEEPQNLIKQNCELFEQLGEYKFQNALLVRYTKKVPQVSTPTLVEVSRNLGKVGSKCCKHPEAKRMPCAEDYLSVVLNQLCVLHEKTPVSDRVTKCCTESLVNRRPCFSALEVDETYVPKEFNAETFTFHADICTLSEKERQIKKQTALVELVKHKPKATKEQLKAVMDDFFVEKCCKADDKETCFAEEGKKLVSQLGLGGGGSCQDGRMGFC

SEQ ID NO: 17 - skipped

SEQ ID NO: 18 - protein, 213 aa, synthetic construct
VEEPQNLIKQNCELFEQLGEYKFQNALLVRYTKKVPQVSTPTLVEVSRNLGKVGSKCCKHPEAKRMPCAEDYLSVVLNQLCVLHEKTPVSDRVTKCCTESLVNRRPCFSALEVDETYVPKEFNAETFTFHADICTLSEKERQIKKQTALVELVKHKPKATKEQLKAVMDDFAAFVEKCCKADDKETCFAEEGKKLVAASQAALGLGGGGSRGD

SEQ ID NO: 19 - protein, 221 aa, synthetic construct
RGDGGGGSVEEPQNLIKQNCELFEQLGEYKFQNALLVRYTKKVPQVSTPTLVEVSRNLGKVGSKCCKHPEAKRMPCAEDYLSVVLNQLCVLHEKTPVSDRVTKCCTESLVNRRPCFSALEVDETYVPKEFNAETFTFHADICTLSEKERQIKKQTALVELVKHKPKATKEQLKAVMDDFAAFVEKCCKADDKETCFAEEGKKLVAASQAALGLGGGGSRGD

SEQ ID NO: 20 - protein, 439 aa, synthetic construct
RGDGGGGSVEEPQNLIKQNCELFEQLGEYKFQNALLVRYTKKVPQVSTPTLVEVSRNLGKVGSKCCKHPEAKRMPCAEDYLSVVLNQLCVLHEKTPVSDRVTKCCTESLVNRRPCFSALEVDETYVPKEFNAETFTFHADICTLSEKERQIKKQTALVELVKHKPKATKEQLKAVMDDFAAFVEKCCKADDKETCFAEEGKKLVAASQAALGLGGGGSRGDGGGGSVEEPQNLIKQNCELFEQLGEYKFQNALLVRYTKKVPQVSTPTLVEVSRNLGKVGSKCCKHPEAKRMPCAEDYLSVVLNQLCVLHEKTPVSDRVTKCCTESLVNRRPCFSALEVDETYVPKEFNAETFTFHADICTLSEKERQIKKQTALVELVKHKPKATKEQLKAVMDDFAAFVEKCCKADDKETCFAEEGKKLVAASQAALGLGGGGSRGD